European Patent Application EP 4 461 807 A1, published November 13, 2024. Title: Sheet-shaped cell culture for treating liver dysfunction. Applicant: OSAKA UNIVERSITY. The sequence listing filed with the application follows.

SEQUENCE LISTING (8 sequences)

SEQ ID NO: 1 - DNA, 20 bp, synthetic construct
  misc_feature 1..20: note = VEGF F
  source 1..20: mol_type = other DNA
gaaggagagcagaagtccca

SEQ ID NO: 2 - DNA, 20 bp, synthetic construct
  misc_feature 1..20: note = VEGF R
  source 1..20: mol_type = other DNA
acacaggacggcttgaagat

SEQ ID NO: 3 - DNA, 20 bp, synthetic construct
  misc_feature 1..20: note = HGF F
  source 1..20: mol_type = other DNA
tgacctgcaatggtgaaagc

SEQ ID NO: 4 - DNA, 20 bp, synthetic construct
  misc_feature 1..20: note = HGF R
  source 1..20: mol_type = other DNA
gggtcaagagtgtagcacca

SEQ ID NO: 5 - DNA, 21 bp, synthetic construct
  misc_feature 1..21: note = Alpha-SMA F
  source 1..21: mol_type = other DNA
gtcccagacatcagggagtaa

SEQ ID NO: 6 - DNA, 21 bp, synthetic construct
  misc_feature 1..21: note = Alpha-SMA R
  source 1..21: mol_type = other DNA
tcggatacttcagcgtcagga

SEQ ID NO: 7 - DNA, 19 bp, synthetic construct
  misc_feature 1..19: note = Type I collagen alpha 1 F
  source 1..19: mol_type = other DNA
gctcctcttaggggccact

SEQ ID NO: 8 - DNA, 19 bp, synthetic construct
  misc_feature 1..19: note = Type I collagen alpha 1 R
  source 1..19: mol_type = other DNA
ccacgtctcaccattgggg